European Patent Application EP 4 410 823 A1, published August 7, 2024. Title: Composition for raising fish, and Compotision for prevention or treatment of fish diseases. Applicant: 住友化学株式会社. Application JP. The sequence listing filed with the application follows.

SEQUENCE LISTING (4 sequences)

SEQ ID NO: 1 - protein, 53 aa, Lactococcus lactis
  MOD_RES 1: note = FORMYLATION
  source 1..53: note = NITE BP-03536
MAGFLKVVQLLAKYGSKAVQWAWANKGKILDWLNAGQAIDWVVSKIKQILGIK

SEQ ID NO: 2 - DNA, 162 bp, Lactococcus lactis
  source 1..162: mol_type = genomic DNA; note = NITE BP-03536
atggcagggtttttaaaagtagttcaattactagctaaatatggttctaaagctgtacaatgggcttgggcaaacaagggtaagattttagattggcttaatgcaggtcaggctattgattgggtagtttcgaaaattaagcaaattttaggtattaagtaa

SEQ ID NO: 3 - protein, 53 aa, Lactococcus lactis
  MOD_RES 1: note = FORMYLATION
MAGFLKVVQILAKYGSKAVQWAWANKGKILDWINAGQAIDWVVEKIKQILGIK

SEQ ID NO: 4 - protein, 53 aa, Curtobacterium
MAVFARILQLLAKYGARAVNWAKANIQRVLNWINAGQAIDWIVSKIKQILGIR